European Patent Application EP 4 520 770 A1, published March 12, 2025. Title: ANTI-CD300C ANTIBODY OR ANTIGEN BINDING FRAGMENT OF THE SAME AND USES THEREOF FOR PREVENTING OR TREATING DEGENERATIVE BRAIN DISEASES. Applicant: CentricsBio, Inc. Application KR. The sequence listing filed with the application follows.

SEQUENCE LISTING (402 sequences)

SEQ ID NO: 1 - DNA, 30 bp, synthetic construct
  source 1..30: mol_type = other DNA
ttcagccgctatgccatgacctgggttcgc

SEQ ID NO: 2 - DNA, 45 bp, synthetic construct
  source 1..45: mol_type = other DNA
agcagcatgagcggcaccggcggcaccacctattatgccgatagc

SEQ ID NO: 3 - DNA, 36 bp, synthetic construct
  source 1..36: mol_type = other DNA
tactgtgcccgcggcgcctatggctttgatcattgg

SEQ ID NO: 4 - DNA, 41 bp, synthetic construct
  source 1..41: mol_type = other DNA
tgccgcgccagccagagcatcggcaactatctgaactggta

SEQ ID NO: 5 - DNA, 36 bp, synthetic construct
  source 1..36: mol_type = other DNA
ctgatctatgatgccagcaacctggaaaccggcatc

SEQ ID NO: 6 - DNA, 45 bp, synthetic construct
  source 1..45: mol_type = other DNA
tattattgtcagcagagtagcgccatcccttataccttcggtcag

SEQ ID NO: 7 - protein, 12 aa, synthetic construct
FTFSRYAMTWVR

SEQ ID NO: 8 - protein, 13 aa, synthetic construct
SMSGTGGTTYYAD

SEQ ID NO: 9 - protein, 12 aa, synthetic construct
YCARGAYGFDHW

SEQ ID NO: 10 - protein, 13 aa, synthetic construct
CRASQSIGNYLNW

SEQ ID NO: 11 - protein, 10 aa, synthetic construct
DASNLETGIP

SEQ ID NO: 12 - protein, 12 aa, synthetic construct
YCQQSSAIPYTF

SEQ ID NO: 13 - DNA, 30 bp, synthetic construct
  source 1..30: mol_type = other DNA
ttcagcagctatggcatgcattgggttcgc

SEQ ID NO: 14 - DNA, 45 bp, synthetic construct
  source 1..45: mol_type = other DNA
agcgccatcagcggcagcggcaccagcatctattatgccgatagc

SEQ ID NO: 15 - DNA, 36 bp, synthetic construct
  source 1..36: mol_type = other DNA
tactgtgcccgcggcggcaccgcctttgattattgg

SEQ ID NO: 16 - DNA, 39 bp, synthetic construct
  source 1..39: mol_type = other DNA
tgccgcgccagccagagatcagacaactatctggcctgg

SEQ ID NO: 17 - DNA, 36 bp, synthetic construct
  source 1..36: mol_type = other DNA
ctgatctatgatgccagcaaccgcgccaccggcatc

SEQ ID NO: 18 - DNA, 45 bp, synthetic construct
  source 1..45: mol_type = other DNA
tattattgtcagcagagctatagcaccccttttaccttcggtcag

SEQ ID NO: 19 - protein, 12 aa, synthetic construct
FTFSSYGMHWVR

SEQ ID NO: 20 - protein, 13 aa, synthetic construct
AISGSGTSIYYAD

SEQ ID NO: 21 - protein, 12 aa, synthetic construct
YCARGGTAFDYW

SEQ ID NO: 22 - protein, 13 aa, synthetic construct
CRASQRSDNYLAW

SEQ ID NO: 23 - protein, 10 aa, synthetic construct
DASNRATGIP

SEQ ID NO: 24 - protein, 12 aa, synthetic construct
YCQQSYSTPFTF

SEQ ID NO: 25 - DNA, 30 bp, synthetic construct
  source 1..30: mol_type = other DNA
ttcagcagctatgccatcagctgggttcgc

SEQ ID NO: 26 - DNA, 45 bp, synthetic construct
  source 1..45: mol_type = other DNA
agcgccaccagcggcagcggccgcgccacctattatgccgatagc

SEQ ID NO: 27 - DNA, 45 bp, synthetic construct
  source 1..45: mol_type = other DNA
tactgtgcgcgcgatacctggtgggaaggctattttgatctgtgg

SEQ ID NO: 28 - DNA, 36 bp, synthetic construct
  source 1..36: mol_type = other DNA
tgccaggccagccatatcagcacccatctgaactgg

SEQ ID NO: 29 - DNA, 36 bp, synthetic construct
  source 1..36: mol_type = other DNA
ctgatctatggcgccagcagccgcgccaccggcatc

SEQ ID NO: 30 - DNA, 45 bp, synthetic construct
  source 1..45: mol_type = other DNA
tattattgtcagcagtataacacctatcctcctaccttcggtcag

SEQ ID NO: 31 - protein, 12 aa, synthetic construct
FTFSSYAISWVR

SEQ ID NO: 32 - protein, 13 aa, synthetic construct
ATSGSGRATYYAD

SEQ ID NO: 33 - protein, 15 aa, synthetic construct
YCARDTWWEGYFDLW

SEQ ID NO: 34 - protein, 12 aa, synthetic construct
CQASHISTHLNW

SEQ ID NO: 35 - protein, 10 aa, synthetic construct
GASSRATGIP

SEQ ID NO: 36 - protein, 12 aa, synthetic construct
YCQQYNTYPPTF

SEQ ID NO: 37 - DNA, 33 bp, synthetic construct
  source 1..33: mol_type = other DNA
accttcggcagcaactatatgagctgggttcgc

SEQ ID NO: 38 - DNA, 33 bp, synthetic construct
  source 1..33: mol_type = other DNA
atcagcggcagcggcaccagcacctattatgcc

SEQ ID NO: 39 - DNA, 27 bp, synthetic construct
  source 1..27: mol_type = other DNA
cgcggcatgtggggcatggatgtgtgg

SEQ ID NO: 40 - DNA, 27 bp, synthetic construct
  source 1..27: mol_type = other DNA
ggcaaacatcggcacaccgtgaactgg

SEQ ID NO: 41 - DNA, 30 bp, synthetic construct
  source 1..30: mol_type = other DNA
ctggatagcgaacgccctagcggcgtacct

SEQ ID NO: 42 - DNA, 27 bp, synthetic construct
  source 1..27: mol_type = other DNA
tatgatagcagcagcgtggtgtttggt

SEQ ID NO: 43 - protein, 12 aa, synthetic construct
FTFGSNYMSWVR

SEQ ID NO: 44 - protein, 13 aa, synthetic construct
TISGSGTSTYYAD

SEQ ID NO: 45 - protein, 12 aa, synthetic construct
YCARGMWGMDVW

SEQ ID NO: 46 - protein, 11 aa, synthetic construct
CTGKHRHTVNW

SEQ ID NO: 47 - protein, 10 aa, synthetic construct
LDSERPSGVP

SEQ ID NO: 48 - protein, 12 aa, synthetic construct
YCQSYDSSSVVF

SEQ ID NO: 49 - DNA, 33 bp, synthetic construct
  source 1..33: mol_type = other DNA
accttcagcagctatgccatgcattgggttcgc

SEQ ID NO: 50 - DNA, 33 bp, synthetic construct
  source 1..33: mol_type = other DNA
atcagcggcggcggctatggcacctattatgcc

SEQ ID NO: 51 - DNA, 30 bp, synthetic construct
  source 1..30: mol_type = other DNA
cgcagcaccgtgtgggcctttgatatctgg

SEQ ID NO: 52 - DNA, 30 bp, synthetic construct
  source 1..30: mol_type = other DNA
ggcaacaacatcggcagcaaaagcgtgcat

SEQ ID NO: 53 - DNA, 30 bp, synthetic construct
  source 1..30: mol_type = other DNA
gatgtgagcaaacgccctagcgagcgtcct

SEQ ID NO: 54 - DNA, 30 bp, synthetic construct
  source 1..30: mol_type = other DNA
tttgatagcagcggcacctggatctttggt

SEQ ID NO: 55 - protein, 12 aa, synthetic construct
FTFSSYAMHWVR

SEQ ID NO: 56 - protein, 13 aa, synthetic construct
SISGGGYGTYYAD

SEQ ID NO: 57 - protein, 13 aa, synthetic construct
YCARSTVWAFDIW

SEQ ID NO: 58 - protein, 13 aa, synthetic construct
CSGNNIGSKSVHW

SEQ ID NO: 59 - protein, 11 aa, synthetic construct
DVSKRPSERPD

SEQ ID NO: 60 - protein, 13 aa, synthetic construct
YCQSFDSSGTWIF

SEQ ID NO: 61 - DNA, 27 bp, synthetic construct
  source 1..27: mol_type = other DNA
agcagctacggtatgcattgggtcaga

SEQ ID NO: 62 - DNA, 39 bp, synthetic construct
  source 1..39: mol_type = other DNA
gcaattagcggtagcggtggtagcacttactacgcagac

SEQ ID NO: 63 - DNA, 45 bp, synthetic construct
  source 1..45: mol_type = other DNA
tgcgcagtcagtggtgcaggtcgtggtttcttcgactactgggga

SEQ ID NO: 64 - DNA, 39 bp, synthetic construct
  source 1..39: mol_type = other DNA
tgcagcggtagcagcagcaacattggtagcaactacgtg

SEQ ID NO: 65 - DNA, 24 bp, synthetic construct
  source 1..24: mol_type = other DNA
gacaacaagcgtcctagtggtgtg

SEQ ID NO: 66 - DNA, 33 bp, synthetic construct
  source 1..33: mol_type = other DNA
tgcagcagctacactagcagcagcactgtgatc

SEQ ID NO: 67 - protein, 12 aa, synthetic construct
FTFSSYGMHWVR

SEQ ID NO: 68 - protein, 13 aa, synthetic construct
AISGSGGSTYYAD

SEQ ID NO: 69 - protein, 15 aa, synthetic construct
YCAVSGAGRGFFDYW

SEQ ID NO: 70 - protein, 15 aa, synthetic construct
CSGSSSNIGSNYVYW

SEQ ID NO: 71 - protein, 10 aa, synthetic construct
EDNKRPSGVP

SEQ ID NO: 72 - protein, 13 aa, synthetic construct
YCSSYTSSSTVIF

SEQ ID NO: 73 - DNA, 27 bp, synthetic construct
  source 1..27: mol_type = other DNA
agccgctacgcaatgagctgggtcaga

SEQ ID NO: 74 - DNA, 39 bp, synthetic construct; identical to SEQ ID NO: 62
  source 1..39: mol_type = other DNA

SEQ ID NO: 75 - DNA, 39 bp, synthetic construct
  source 1..39: mol_type = other DNA
tgcgcacgtagcagccagggtatcttcgacatctgggga

SEQ ID NO: 76 - DNA, 33 bp, synthetic construct
  source 1..33: mol_type = other DNA
tgcagtggtaacaatatcggtactagacgcgtg

SEQ ID NO: 77 - DNA, 24 bp, synthetic construct
  source 1..24: mol_type = other DNA
aagaacaaccgtcctagtggtgtg

SEQ ID NO: 78 - DNA, 39 bp, synthetic construct
  source 1..39: mol_type = other DNA
tgcgcagcatgggacgacagcctgagcggtcctgtgttc

SEQ ID NO: 79 - protein, 12 aa, synthetic construct
FTFSRYAMSWVR

SEQ ID NO: 80 - protein, 13 aa, synthetic construct
AISGSGGSTYYAD

SEQ ID NO: 81 - protein, 13 aa, synthetic construct
YCARSSQGIFDIW

SEQ ID NO: 82 - protein, 13 aa, synthetic construct
CSGNNIGTRRVHW

SEQ ID NO: 83 - protein, 10 aa, synthetic construct
SKNNRPSGVP

SEQ ID NO: 84 - protein, 14 aa, synthetic construct
YCAAWDDSLSGPVF

SEQ ID NO: 85 - DNA, 27 bp, synthetic construct
  source 1..27: mol_type = other DNA
agcagctacgcaatgagctgggtcaga

SEQ ID NO: 86 - DNA, 39 bp, synthetic construct; identical to SEQ ID NO: 62
  source 1..39: mol_type = other DNA

SEQ ID NO: 87 - DNA, 42 bp, synthetic construct
  source 1..42: mol_type = other DNA
tgcgcacgtagcggtcgttacgcagacttgacatctggggga

SEQ ID NO: 88 - DNA, 39 bp, synthetic construct
  source 1..39: mol_type = other DNA
tgcagcggtagcaacagcaacatcggtaacaactacgtg

SEQ ID NO: 89 - DNA, 24 bp, synthetic construct
  source 1..24: mol_type = other DNA
aacaacaagcgtcctagtggtgtg

SEQ ID NO: 90 - DNA, 36 bp, synthetic construct
  source 1..36: mol_type = other DNA
tgcagcagctacactagcagcagcactgtgatgttc

SEQ ID NO: 91 - protein, 12 aa, synthetic construct
FTFSSYAMSWVR

SEQ ID NO: 92 - protein, 13 aa, synthetic construct
AISGSGGSTYYAD

SEQ ID NO: 93 - protein, 14 aa, synthetic construct
YCARSGRYADLTSG

SEQ ID NO: 94 - protein, 15 aa, synthetic construct
CSGSNSNIGNNYVSW

SEQ ID NO: 95 - protein, 10 aa, synthetic construct
DNNKRPSGVP

SEQ ID NO: 96 - protein, 13 aa, synthetic construct
YCSSYTSSSTVMF

SEQ ID NO: 97 - DNA, 27 bp, synthetic construct
  source 1..27: mol_type = other DNA
agcagctactactggagctgggtcaga

SEQ ID NO: 98 - DNA, 39 bp, synthetic construct; identical to SEQ ID NO: 62
  source 1..39: mol_type = other DNA

SEQ ID NO: 99 - DNA, 39 bp, synthetic construct
  source 1..39: mol_type = other DNA
tgcgcacgtatcgacgtgtacggtttcgacatctgggga

SEQ ID NO: 100 - DNA, 39 bp, synthetic construct
  source 1..39: mol_type = other DNA
tgcagcggtagcactagcaacatcggtactaactacgtg

SEQ ID NO: 101 - DNA, 24 bp, synthetic construct
  source 1..24: mol_type = other DNA
aacaacaaccgtcctagtggtgtg

SEQ ID NO: 102 - DNA, 33 bp, synthetic construct
  source 1..33: mol_type = other DNA
tgccagacttgggacagcagcactgacgtagtg

SEQ ID NO: 103 - protein, 12 aa, synthetic construct
FTFSSYYWSWVR

SEQ ID NO: 104 - protein, 13 aa, synthetic construct
AISGSGGSTYYAD

SEQ ID NO: 105 - protein, 13 aa, synthetic construct
YCARIDVYGFDIW

SEQ ID NO: 106 - protein, 15 aa, synthetic construct
CSGSTSNIGTNYVYW

SEQ ID NO: 107 - protein, 10 aa, synthetic construct
DNNNRPSGVP

SEQ ID NO: 108 - protein, 13 aa, synthetic construct
YCQTWDSSTDVVF

SEQ ID NO: 109 - DNA, 31 bp, synthetic construct
  source 1..31: mol_type = other DNA
tcagcagctacggtatgcattgggtcagaca

SEQ ID NO: 110 - DNA, 43 bp, synthetic construct
  source 1..43: mol_type = other DNA
ctgcaattagcggtagcggtggtagcacttactacgcagacag

SEQ ID NO: 111 - DNA, 40 bp, synthetic construct
  source 1..40: mol_type = other DNA
actgcgcaagcggttacggtctgatggacgtgtggggaca

SEQ ID NO: 112 - DNA, 43 bp, synthetic construct
  source 1..43: mol_type = other DNA
gctgcactcgtagcagcggtatcatcgcaagcaactacgtgca

SEQ ID NO: 113 - DNA, 27 bp, synthetic construct
  source 1..27: mol_type = other DNA
cgcaacaaccagcgccctagtggtgtg

SEQ ID NO: 114 - DNA, 40 bp, synthetic construct
  source 1..40: mol_type = other DNA
actgcagcagctacgcaggtaacaacaacctggtgttcgg

SEQ ID NO: 115 - protein, 12 aa, synthetic construct
FTFSSYGMHWVR

SEQ ID NO: 116 - protein, 13 aa, synthetic construct
AISGSGGSTYYAD

SEQ ID NO: 117 - protein, 12 aa, synthetic construct
YCASGYGLMDVW

SEQ ID NO: 118 - protein, 15 aa, synthetic construct
CTRSSGIIASNYVQW

SEQ ID NO: 119 - protein, 10 aa, synthetic construct
RNNQRPSGVP

SEQ ID NO: 120 - protein, 13 aa, synthetic construct
YCSSYAGNNNLVF

SEQ ID NO: 121 - DNA, 30 bp, synthetic construct
  source 1..30: mol_type = other DNA
ttcagcacctatggcatgcattgggttcgc

SEQ ID NO: 122 - DNA, 42 bp, synthetic construct
  source 1..42: mol_type = other DNA
agcgccatcagcggcagcggcggcagcacctattatgccgat

SEQ ID NO: 123 - DNA, 36 bp, synthetic construct
  source 1..36: mol_type = other DNA
tactgtgcccgcggcctgagcggccttgattattgg

SEQ ID NO: 124 - DNA, 39 bp, synthetic construct
  source 1..39: mol_type = other DNA
tgccgctccagccagggcatcaccaactatctggcctgg

SEQ ID NO: 125 - DNA, 36 bp, synthetic construct; identical to SEQ ID NO: 17
  source 1..36: mol_type = other DNA

SEQ ID NO: 126 - DNA, 45 bp, synthetic construct
  source 1..45: mol_type = other DNA
tattattgtcagcagagctatagcacccctctgaccttcggtcag

SEQ ID NO: 127 - protein, 12 aa, synthetic construct
FTFSTYGMHWVR

SEQ ID NO: 128 - protein, 13 aa, synthetic construct
AISGSGGSTYYAD

SEQ ID NO: 129 - protein, 12 aa, synthetic construct
YCARGLSGLDYW

SEQ ID NO: 130 - protein, 13 aa, synthetic construct
CRSSQGITNYLAW

SEQ ID NO: 131 - protein, 10 aa, synthetic construct
DASNRATGIP

SEQ ID NO: 132 - protein, 12 aa, synthetic construct
YCQQSYSTPLTF

SEQ ID NO: 133 - DNA, 34 bp, synthetic construct
  source 1..34: mol_type = other DNA
ccttcagcagctatgccatgcattgggttcgcca

SEQ ID NO: 134 - DNA, 49 bp, synthetic construct
  source 1..49: mol_type = other DNA
tgagcgccatcagcggcagcggcggcgatacctatcatgccgatagcgt

SEQ ID NO: 135 - DNA, 40 bp, synthetic construct
  source 1..40: mol_type = other DNA
actactgtacccgcggcctgagcggctttgattattgggg

SEQ ID NO: 136 - DNA, 43 bp, synthetic construct
  source 1..43: mol_type = other DNA
catgccgcgccagccagagcatcagcagctatctgaactggta

SEQ ID NO: 137 - DNA, 40 bp, synthetic construct
  source 1..40: mol_type = other DNA
tgctgatctatgatgccagcaaccgcgcccctggcatccc

SEQ ID NO: 138 - DNA, 49 bp, synthetic construct
  source 1..49: mol_type = other DNA
tgtattattgtcagcagagctatagcatccctatcaccttcggtcaggg

SEQ ID NO: 139 - protein, 12 aa, synthetic construct
FTFSSYAMHWVR

SEQ ID NO: 140 - protein, 13 aa, synthetic construct
AISGSGGDTYHAD

SEQ ID NO: 141 - protein, 12 aa, synthetic construct
YCTRGLSGFDYW

SEQ ID NO: 142 - protein, 13 aa, synthetic construct
CRASQSISSYLNW

SEQ ID NO: 143 - protein, 10 aa, synthetic construct
DASNRAPGIP

SEQ ID NO: 144 - protein, 12 aa, synthetic construct
YCQQSYSIPITF

SEQ ID NO: 145 - DNA, 30 bp, synthetic construct
  source 1..30: mol_type = other DNA
ttcagcgattatgccatgagctgggttcgc

SEQ ID NO: 146 - DNA, 42 bp, synthetic construct
  source 1..42: mol_type = other DNA
agcatcagcagcagcagcagctatatctactataccgatagc

SEQ ID NO: 147 - DNA, 36 bp, synthetic construct
  source 1..36: mol_type = other DNA
tactgtgcccgcggcggctatggctttgattattgg

SEQ ID NO: 148 - DNA, 39 bp, synthetic construct
  source 1..39: mol_type = other DNA
tgccgcgccagccagagcatcagcagctatctgaactgg

SEQ ID NO: 149 - DNA, 36 bp, synthetic construct
  source 1..36: mol_type = other DNA
ctgatctatagcgccagcagccgcccacagggcatc

SEQ ID NO: 150 - DNA, 45 bp, synthetic construct
  source 1..45: mol_type = other DNA
tattattgtcagcagtatgatgatctgccttttaccttcggtcag

SEQ ID NO: 151 - protein, 12 aa, synthetic construct
FTFSDYAMSWVR

SEQ ID NO: 152 - protein, 13 aa, synthetic construct
SISSSSSYIYYTD

SEQ ID NO: 153 - protein, 12 aa, synthetic construct
YCARGGYGFDYW

SEQ ID NO: 154 - protein, 13 aa, synthetic construct
CRASQSISSYLNW

SEQ ID NO: 155 - protein, 10 aa, synthetic construct
SASSRPQGIP

SEQ ID NO: 156 - protein, 12 aa, synthetic construct
YCQQYDDLPFTF

SEQ ID NO: 157 - DNA, 34 bp, synthetic construct
  source 1..34: mol_type = other DNA
ccttcagcaactttgcgatcgcctgggttcgcca

SEQ ID NO: 158 - DNA, 46 bp, synthetic construct
  source 1..46: mol_type = other DNA
gcgccatcagcggccgcggcaccagcacctattatgccgatagcgt

SEQ ID NO: 159 - DNA, 40 bp, synthetic construct
  source 1..40: mol_type = other DNA
actactgtgcccgcggcgtgagcggctttgatagctgggg

SEQ ID NO: 160 - DNA, 43 bp, synthetic construct
  source 1..43: mol_type = other DNA
catgccgcgccagccagagcatcagcagccatctggcctggta

SEQ ID NO: 161 - DNA, 40 bp, synthetic construct
  source 1..40: mol_type = other DNA
tgctgatctatgataccagcaaccgcgccaccggcatccc

SEQ ID NO: 162 - DNA, 49 bp, synthetic construct
  source 1..49: mol_type = other DNA
tgtactattgtcagcagagctatagcaccccttttaccttcggtcaggg

SEQ ID NO: 163 - protein, 12 aa, synthetic construct
FTFSNFAIAWVR

SEQ ID NO: 164 - protein, 13 aa, synthetic construct
AISGRGTSTYYAD

SEQ ID NO: 165 - protein, 12 aa, synthetic construct
YCARGVSGFDSW

SEQ ID NO: 166 - protein, 13 aa, synthetic construct
CRASQSISSHLAW

SEQ ID NO: 167 - protein, 10 aa, synthetic construct
DTSNRATGIP

SEQ ID NO: 168 - protein, 12 aa, synthetic construct
YCQQSYSTPFTF

SEQ ID NO: 169 - DNA, 34 bp, synthetic construct; identical to SEQ ID NO: 133
  source 1..34: mol_type = other DNA

SEQ ID NO: 170 - DNA, 49 bp, synthetic construct
  source 1..49: mol_type = other DNA
tgagcgccatcaacggcagcggcggcagcacctattatgccgatagcgt

SEQ ID NO: 171 - DNA, 43 bp, synthetic construct
  source 1..43: mol_type = other DNA
actactgtgcccgcggcctgcagggctttgattattggggaca

SEQ ID NO: 172 - DNA, 43 bp, synthetic construct
  source 1..43: mol_type = other DNA
catgccaggccagccaggatatcaccaactatctgaactggta

SEQ ID NO: 173 - DNA, 40 bp, synthetic construct
  source 1..40: mol_type = other DNA
tgctgatctatgatgccagcagcctggaaaccggcatccc

SEQ ID NO: 174 - DNA, 49 bp, synthetic construct
  source 1..49: mol_type = other DNA
tgtattattgtcagcagagctatagcacccctatcaccttcggtcaggg

SEQ ID NO: 175 - protein, 12 aa, synthetic construct
FTFSSYAMHWVR

SEQ ID NO: 176 - protein, 13 aa, synthetic construct
AINGSGGSTYYAD

SEQ ID NO: 177 - protein, 12 aa, synthetic construct
YCARGLQGFDYW

SEQ ID NO: 178 - protein, 13 aa, synthetic construct
CQASQDITNYLNW

SEQ ID NO: 179 - protein, 10 aa, synthetic construct
DASSLETGIP

SEQ ID NO: 180 - protein, 12 aa, synthetic construct
YCQQSYSTPITF

SEQ ID NO: 181 - DNA, 34 bp, synthetic construct
  source 1..34: mol_type = other DNA
ccttcagcagctatgccatgagctgggttcgcca

SEQ ID NO: 182 - DNA, 49 bp, synthetic construct
  source 1..49: mol_type = other DNA
tgagcgccatcaacggcagcggcggcagcaccctgtatgccgatagcgt

SEQ ID NO: 183 - DNA, 40 bp, synthetic construct; identical to SEQ ID NO: 159
  source 1..40: mol_type = other DNA

SEQ ID NO: 184 - DNA, 43 bp, synthetic construct
  source 1..43: mol_type = other DNA
catgccgcatcagccagagcatcagcagctatctgaactggta

SEQ ID NO: 185 - DNA, 40 bp, synthetic construct
  source 1..40: mol_type = other DNA
tgctgatctatgatgccagcctgcgcgccaccggcatccc

SEQ ID NO: 186 - DNA, 49 bp, synthetic construct
  source 1..49: mol_type = other DNA
tgtattattgtcagcagagctataaaacccctatcaccttcggtcaggg

SEQ ID NO: 187 - protein, 12 aa, synthetic construct
FTFSSYAMSWVR

SEQ ID NO: 188 - protein, 13 aa, synthetic construct
AINGSGGSTLYAD

SEQ ID NO: 189 - protein, 12 aa, synthetic construct
YCARGVSGFDSW

SEQ ID NO: 190 - protein, 13 aa, synthetic construct
CRISQSISSYLNW

SEQ ID NO: 191 - protein, 10 aa, synthetic construct
DASLRATGIP

SEQ ID NO: 192 - protein, 13 aa, synthetic construct
YYCQQSYKTPITF

SEQ ID NO: 193 - DNA, 34 bp, synthetic construct
  source 1..34: mol_type = other DNA
ccttcagcagctattattggagctgggttcgcca

SEQ ID NO: 194 - DNA, 49 bp, synthetic construct
  source 1..49: mol_type = other DNA
tgagcaccatcaccggcagcggcggcagcaccgattatgccaacagcgt

SEQ ID NO: 195 - DNA, 40 bp, synthetic construct
  source 1..40: mol_type = other DNA
actactgtgccaccggcggcggcatctttgactattgggg

SEQ ID NO: 196 - DNA, 43 bp, synthetic construct
  source 1..43: mol_type = other DNA
catgccaggccagccagaccatcagcaactatctgaactggta

SEQ ID NO: 197 - DNA, 40 bp, synthetic construct
  source 1..40: mol_type = other DNA
tgctgatctatgatgccagcaaccgcgccaccggcatccc

SEQ ID NO: 198 - DNA, 49 bp, synthetic construct
  source 1..49: mol_type = other DNA
tgtattattgtcagcagtacaacagctatcctcctagcttcggtcaggg

SEQ ID NO: 199 - protein, 12 aa, synthetic construct
FTFSSYYWSWVR

SEQ ID NO: 200 - protein, 13 aa, synthetic construct
TITGSGGSTDYAN

SEQ ID NO: 201 - protein, 12 aa, synthetic construct
YCATGGGIFDYW

SEQ ID NO: 202 - protein, 13 aa, synthetic construct
CQASQTISNYLNW

SEQ ID NO: 203 - protein, 10 aa, synthetic construct
DASNRATGIP

SEQ ID NO: 204 - protein, 12 aa, synthetic construct
YCQQYNSYPPSF

SEQ ID NO: 205 - DNA, 34 bp, synthetic construct
  source 1..34: mol_type = other DNA
tcaccttcagcgattatcatatgcattgggttcg

SEQ ID NO: 206 - DNA, 34 bp, synthetic construct
  source 1..34: mol_type = other DNA
tcagcagcagcggcggctatacctattatgccga

SEQ ID NO: 207 - DNA, 34 bp, synthetic construct
  source 1..34: mol_type = other DNA
cccgatcgatacgcctgcctctggattattgggg

SEQ ID NO: 208 - DNA, 37 bp, synthetic construct
  source 1..37: mol_type = other DNA
gcggcaacaacatcggcagcaaaggcgtgcattggta

SEQ ID NO: 209 - DNA, 34 bp, synthetic construct
  source 1..34: mol_type = other DNA
atgaagatagcaaacgccctagcggcgtgcgtga

SEQ ID NO: 210 - DNA, 34 bp, synthetic construct
  source 1..34: mol_type = other DNA
gctatgatagcaccaaaggcgtggtgtttggtgg

SEQ ID NO: 211 - protein, 12 aa, synthetic construct
FTFSDYHMHWVR

SEQ ID NO: 212 - protein, 13 aa, synthetic construct
TISSSGGYTYYAE

SEQ ID NO: 213 - protein, 13 aa, synthetic construct
YCARSIRLPLDYW

SEQ ID NO: 214 - protein, 13 aa, synthetic construct
CSGNNIGSKGVHW

SEQ ID NO: 215 - protein, 10 aa, synthetic construct
EDSKRPSGVR

SEQ ID NO: 216 - protein, 13 aa, synthetic construct
YCQSYDSTKGVVF

SEQ ID NO: 217 - DNA, 34 bp, synthetic construct
  source 1..34: mol_type = other DNA
tcagcagctacggtatgcattgggtcagacaggc

SEQ ID NO: 218 - DNA, 43 bp, synthetic construct; identical to SEQ ID NO: 110
  source 1..43: mol_type = other DNA

SEQ ID NO: 219 - DNA, 40 bp, synthetic construct
  source 1..40: mol_type = other DNA
actgcgtgcgtggttacggtgcaatggacgtgtggggaca

SEQ ID NO: 220 - DNA, 43 bp, synthetic construct
  source 1..43: mol_type = other DNA
gctgcactcgtagcagcggtagcatcgcaagcaactacgtgca

SEQ ID NO: 221 - DNA, 31 bp, synthetic construct
  source 1..31: mol_type = other DNA
accgcaacaaccagcgccctagtggtgtgcc

SEQ ID NO: 222 - DNA, 40 bp, synthetic construct
  source 1..40: mol_type = other DNA
actgcagcagctacactactagcagcactctggtgttcgg

SEQ ID NO: 223 - protein, 12 aa, synthetic construct
FTFSSYGMHWVR

SEQ ID NO: 224 - protein, 13 aa, synthetic construct
AISGSGGSTYYAD

SEQ ID NO: 225 - protein, 12 aa, synthetic construct
YCVRGYGAMDVW

SEQ ID NO: 226 - protein, 15 aa, synthetic construct
CTRSSGSIASNYVQW

SEQ ID NO: 227 - protein, 10 aa, synthetic construct
RNNQRPSGVP

SEQ ID NO: 228 - protein, 13 aa, synthetic construct
YCSSYTTSSTLVF

SEQ ID NO: 229 - DNA, 34 bp, synthetic construct
  source 1..34: mol_type = other DNA
tcagcagctacgcaatgcattgggtcagacaggc

SEQ ID NO: 230 - DNA, 43 bp, synthetic construct; identical to SEQ ID NO: 110
  source 1..43: mol_type = other DNA

SEQ ID NO: 231 - DNA, 40 bp, synthetic construct
  source 1..40: mol_type = other DNA
actgcgcaagcggctacggtctgatggacgtatggggaca

SEQ ID NO: 232 - DNA, 46 bp, synthetic construct
  source 1..46: mol_type = other DNA
gctgcactggtactagcagcgacgtgggtaactacaacctggtgag

SEQ ID NO: 233 - DNA, 31 bp, synthetic construct
  source 1..31: mol_type = other DNA
acagcaacaaccagcgccctagtggtgtgcc

SEQ ID NO: 234 - DNA, 40 bp, synthetic construct
  source 1..40: mol_type = other DNA
actgcagcagctacactggtagcaacgctctgttgttcgg

SEQ ID NO: 235 - protein, 12 aa, synthetic construct
FTFSSYAMHWVR

SEQ ID NO: 236 - protein, 13 aa, synthetic construct
AISGSGGSTYYAD

SEQ ID NO: 237 - protein, 12 aa, synthetic construct
YCASGYGLMDVW

SEQ ID NO: 238 - protein, 16 aa, synthetic construct
CTGTSSDVGNYNLVSW

SEQ ID NO: 239 - protein, 10 aa, synthetic construct
SNNQRPSGVP

SEQ ID NO: 240 - protein, 13 aa, synthetic construct
YCSSYTGSNALLF

SEQ ID NO: 241 - DNA, 31 bp, synthetic construct
  source 1..31: mol_type = other DNA
tcagcagctacgcaatgagctgggtcagaca

SEQ ID NO: 242 - DNA, 43 bp, synthetic construct; identical to SEQ ID NO: 110
  source 1..43: mol_type = other DNA

SEQ ID NO: 243 - DNA, 40 bp, synthetic construct
  source 1..40: mol_type = other DNA
actgcgcacgctggcattacagcttcgactactggggaca

SEQ ID NO: 244 - DNA, 37 bp, synthetic construct
  source 1..37: mol_type = other DNA
gctgccgtggtaacaacatcggtagcaagcgtgtgca

SEQ ID NO: 245 - DNA, 31 bp, synthetic construct
  source 1..31: mol_type = other DNA
acagctacaaccaccgtcctagcggtgtgcc

SEQ ID NO: 246 - DNA, 43 bp, synthetic construct
  source 1..43: mol_type = other DNA
actgcaacacttgggacgacagcctggagggtcctgtgttcgg

SEQ ID NO: 247 - protein, 12 aa, synthetic construct
FTFSSYAMSWVR

SEQ ID NO: 248 - protein, 13 aa, synthetic construct
AISGSGGSTYYAD

SEQ ID NO: 249 - protein, 12 aa, synthetic construct
YCARWHYSFDYW

SEQ ID NO: 250 - protein, 13 aa, synthetic construct
CRGNNIGSKRVHW

SEQ ID NO: 251 - protein, 10 aa, synthetic construct
SYNHRPSGVP

SEQ ID NO: 252 - protein, 14 aa, synthetic construct
YCNTWDDSLEGPVF

SEQ ID NO: 253 - DNA, 31 bp, synthetic construct
  source 1..31: mol_type = other DNA
tcagcggctacgcaatgagctgggtcagaca

SEQ ID NO: 254 - DNA, 43 bp, synthetic construct; identical to SEQ ID NO: 110
  source 1..43: mol_type = other DNA

SEQ ID NO: 255 - DNA, 43 bp, synthetic construct
  source 1..43: mol_type = other DNA
actgcgcacgtagtcctagcggtctgttcgactactggggaca

SEQ ID NO: 256 - DNA, 37 bp, synthetic construct
  source 1..37: mol_type = other DNA
gctgcggtggtaacaacatcggtagcaagcgtgtgca

SEQ ID NO: 257 - DNA, 31 bp, synthetic construct
  source 1..31: mol_type = other DNA
acaacactagcaacaagcatagcggtgtgcc

SEQ ID NO: 258 - DNA, 37 bp, synthetic construct
  source 1..37: mol_type = other DNA
actgcagcagctacctacagcagcactctctgttcgg

SEQ ID NO: 259 - protein, 12 aa, synthetic construct
FTFSGYAMSWVR

SEQ ID NO: 260 - protein, 13 aa, synthetic construct
AISGSGGSTYYAD

SEQ ID NO: 261 - protein, 13 aa, synthetic construct
YCARSPSGLFDYW

SEQ ID NO: 262 - protein, 13 aa, synthetic construct
CGGNNIGSKRVHW

SEQ ID NO: 263 - protein, 10 aa, synthetic construct
NTSNKHSGVP

SEQ ID NO: 264 - protein, 12 aa, synthetic construct
YCSSYLQQHSLF

SEQ ID NO: 265 - DNA, 29 bp, synthetic construct
  source 1..29: mol_type = other DNA
agcagctacgcaatgagctgggtcagaca

SEQ ID NO: 266 - DNA, 43 bp, synthetic construct; identical to SEQ ID NO: 110
  source 1..43: mol_type = other DNA

SEQ ID NO: 267 - DNA, 49 bp, synthetic construct
  source 1..49: mol_type = other DNA
actgcacacgtttcgtgggtgcaatcggtgcattcgactactggggaca

SEQ ID NO: 268 - DNA, 37 bp, synthetic construct
  source 1..37: mol_type = other DNA
gctgcagtggtaacaacatcggtagccgtagcgtgca

SEQ ID NO: 269 - DNA, 31 bp, synthetic construct; identical to SEQ ID NO: 221
  source 1..31: mol_type = other DNA

SEQ ID NO: 270 - DNA, 43 bp, synthetic construct
  source 1..43: mol_type = other DNA
actgcgcagcatgggacgacagcctgagcggtcctgtgttcgg

SEQ ID NO: 271 - protein, 12 aa, synthetic construct
FTFSSYAMSWVR

SEQ ID NO: 272 - protein, 13 aa, synthetic construct
AISGSGGSTYYAD

SEQ ID NO: 273 - protein, 15 aa, synthetic construct
YCTRFVGAIGAFDYW

SEQ ID NO: 274 - protein, 13 aa, synthetic construct
CSGNNIGSRSVHW

SEQ ID NO: 275 - protein, 10 aa, synthetic construct
RNNQRPSGVP

SEQ ID NO: 276 - protein, 14 aa, synthetic construct
YCAAWDDSLSGPVF

SEQ ID NO: 277 - DNA, 31 bp, synthetic construct
  source 1..31: mol_type = other DNA
tcagccattacgcaatgagctgggtcagaca

SEQ ID NO: 278 - DNA, 43 bp, synthetic construct; identical to SEQ ID NO: 110
  source 1..43: mol_type = other DNA

SEQ ID NO: 279 - DNA, 55 bp, synthetic construct
  source 1..55: mol_type = other DNA
actgcgcacgtggttgggacagccctactctgacatacttcgacagctggggaca

SEQ ID NO: 280 - DNA, 43 bp, synthetic construct
  source 1..43: mol_type = other DNA
gctgcagcggtactagcagcaacatcggtaacaacgacgtgag

SEQ ID NO: 281 - DNA, 31 bp, synthetic construct
  source 1..31: mol_type = other DNA
accaggacactaagcgtcctagcggtgtgcc

SEQ ID NO: 282 - DNA, 43 bp, synthetic construct; identical to SEQ ID NO: 270
  source 1..43: mol_type = other DNA

SEQ ID NO: 283 - protein, 12 aa, synthetic construct
FTFSHYAMSWVR

SEQ ID NO: 284 - protein, 13 aa, synthetic construct
AISGSGGSTYYAD

SEQ ID NO: 285 - protein, 17 aa, synthetic construct
YCARGWDSPTLTYFDSW

SEQ ID NO: 286 - protein, 15 aa, synthetic construct
CSGTSSNIGNNDVSW

SEQ ID NO: 287 - protein, 10 aa, synthetic construct
QDTKRPSGVP

SEQ ID NO: 288 - protein, 14 aa, synthetic construct
YCAAWDDSLSGPVF

SEQ ID NO: 289 - DNA, 27 bp, synthetic construct
  source 1..27: mol_type = other DNA
agcagctacggtatgcattgggtcaga

SEQ ID NO: 290 - DNA, 39 bp, synthetic construct
  source 1..39: mol_type = other DNA
gcaatcagcggtagcggtggttacacttactacgcagac

SEQ ID NO: 291 - DNA, 36 bp, synthetic construct
  source 1..36: mol_type = other DNA
tgcgcacgctggcattacagcttcgactactgggga

SEQ ID NO: 292 - DNA, 39 bp, synthetic construct
  source 1..39: mol_type = other DNA
tgcagcggtagcagcagcaacatcggtaacaactacgtg

SEQ ID NO: 293 - DNA, 27 bp, synthetic construct
  source 1..27: mol_type = other DNA
cgcaacaaccagcgccctagtggtgtg

SEQ ID NO: 294 - DNA, 33 bp, synthetic construct
  source 1..33: mol_type = other DNA
tgccagagctacgacaacagcaacgtgctgttc

SEQ ID NO: 295 - protein, 12 aa, synthetic construct
FTFSSYGMHWVR

SEQ ID NO: 296 - protein, 13 aa, synthetic construct
AISGSGGYTYYAD

SEQ ID NO: 297 - protein, 12 aa, synthetic construct
YCARWHYSFDYW

SEQ ID NO: 298 - protein, 15 aa, synthetic construct
CSGSSSNIGNNYVSW

SEQ ID NO: 299 - protein, 10 aa, synthetic construct
RNNQRPSGVP

SEQ ID NO: 300 - protein, 12 aa, synthetic construct
YCQSYDNSNVLF

SEQ ID NO: 301 - DNA, 348 bp, synthetic construct
  source 1..348: mol_type = other DNA
gaagtgcagctgctggaaagtggaggtggactggtgcagcctggcggcagcctgcgcctgagctgtgccgccagcggattcaccttcagccgctatgccatgacctgggttcgccaagcacctggcaaaggcctggaatgggtgagcagcatgagcggcaccggcggcaccacctattatgccgatagcgtgaaaggtcgctttaccatcagccgcgataacagcaaaaacaccctgtatctgcagatgaacagcctgcgcgccgaggacaccgcagtctactactgtgcccgcggcgcctatggctttgatcattggggacaaggtactctggtgaccgtgagcagc

SEQ ID NO: 302 - DNA, 321 bp, synthetic construct
  source 1..321: mol_type = other DNA
gaaatcgtgctgacccagagccctggcaccctgagcctgagccctggcgaacgcgcaacactgtcatgccgcgccagccagagcatcggcaactatctgaactggtatcagcagaaaccaggtcaggctccacgtctgctgatctatgatgccagcaacctggaaaccggcatccctgatcgcttctcaggatctggaagcggtaccgattttaccctgaccatcagccgcctggaacctgaggactttgccgtgtattattgtcagcagagtagcgccatcccttataccttcggtcagggcactaaagtggaaatcaaa

SEQ ID NO: 303 - protein, 116 aa, synthetic construct
EVQLLESGGGLVQPGGSLRLSCAASGFTFSRYAMTWVRQAPGKGLEWVSSMSGTGGTTYYADSVKGRFTISRDNSKNTLYLQMNSLRAEDTAVYYCARGAYGFDHWGQGTLVTVSS

SEQ ID NO: 304 - protein, 107 aa, synthetic construct
EIVLTQSPGTLSLSPGERATLSCRASQSIGNYLNWYQQKPGQAPRLLIYDASNLETGIPDRFSGSGSGTDFTLTISRLEPEDFAVYYCQQSSAIPYTFGQGTKVEIK

SEQ ID NO: 305 - DNA, 348 bp, synthetic construct
  source 1..348: mol_type = other DNA
gaagtgcagctgctggaaagtggaggtggactggtgcagcctggcggcagcctgcgcctgagctgtgccgccagcggattcaccttcagcagctatggcatgcattgggttcgccaagcacctggcaaaggcctggaatgggtgagcgccatcagcggcagcggcaccagcatctattatgccgatagcgtgaaaggccgctttaccatcagccgcgataacagcaaaaacaccctgtatctgcagatgaacagcctgcgcgccgaggacaccgcagtctactactgtgcccgcggcggcaccgcctttgattattggggacaaggtactctggtgaccgtgagcagc

SEQ ID NO: 306 - DNA, 321 bp, synthetic construct
  source 1..321: mol_type = other DNA
gaaatcgtgctgacccagagccctggcaccctgagcctgagccctggcgaacgcgcaacactgtcatgccgcgccagccagagatcagacaactatctggcctggtatcagcagaaaccaggtcaggctccacgtctgctgatctatgatgccagcaaccgcgccaccggcatccctgatcgcttctcaggatctggaagcggtaccgattttaccctgaccatcagccgcctggaacctgaggactttgccgtgtattattgtcagcagagctatagcaccccttttaccttcggtcagggcactaaagtggaaaccaaa

SEQ ID NO: 307 - protein, 116 aa, synthetic construct
EVQLLESGGGLVQPGGSLRLSCAASGFTFSSYGMHWVRQAPGKGLEWVSAISGSGTSIYYADSVKGRFTISRDNSKNTLYLQMNSLRAEDTAVYYCARGGTAFDYWGQGTLVTVSS

SEQ ID NO: 308 - protein, 107 aa, synthetic construct
EIVLTQSPGTLSLSPGERATLSCRASQRSDNYLAWYQQKPGQAPRLLIYDASNRATGIPDRFSGSGSGTDFTLTISRLEPEDFAVYYCQQSYSTPFTFGQGTKVETK

SEQ ID NO: 309 - DNA, 357 bp, synthetic construct
  source 1..357: mol_type = other DNA
cgagtgcagctgctggaaagtggaggtggactggtgcagcctggcggcagcctgcgcctgagctgtgccgccagcggattcaccttcagcagctatgccatcagctgggttcgccaagcacctggcaaaggcctggaatgggtgagcgccaccagcggcagcggccgcgccacctattatgccgatagcgtgaaaggccgctttaccatcagccgcgataacagcaaaaacaccctgtatctgcagatgaacagcctgcgcgccgaggacaccgcagtctactactgtgcgcgcgatacctggtgggaaggctattttgatctgtggggacaaggtactctggtgaccgtgagcagc

SEQ ID NO: 310 - DNA, 318 bp, synthetic construct
  source 1..318: mol_type = other DNA
gaaatcgtgctgacccagagccctggcaccctgagcctgagccctggcgaacgcgcaacactgtcatgccaggccagccatatcagcacccatctgaactggtatcagcagaaaccaggtcaggctccacgtctgctgatctatggcgccagcagccgcgccaccggcatccctgatcgcttctcaggatctggaagcggtaccgattttaccctgaccatcagccgcctggaacctgaggactttgccgtgtattattgtcagcagtataacacctatcctcctaccttcggtcagggcactaaagtggaaatcaaa

SEQ ID NO: 311 - protein, 119 aa, synthetic construct
RVQLLESGGGLVQPGGSLRLSCAASGFTFSSYAISWVRQAPGKGLEWVSATSGSGRATYYADSVKGRFTISRDNSKNTLYLQMNSLRAEDTAVYYCARDTWWEGYFDLWGQGTLVTVSS

SEQ ID NO: 312 - protein, 106 aa, synthetic construct
EIVLTQSPGTLSLSPGERATLSCQASHISTHLNWYQQKPGQAPRLLIYGASSRATGIPDRFSGSGSGTDFTLTISRLEPEDFAVYYCQQYNTYPPTFGQGTKVEIK

SEQ ID NO: 313 - DNA, 348 bp, synthetic construct
  source 1..348: mol_type = other DNA
cgagtgcagctgctggaaagtggaggtggactggtgcagcctggcggcagcctgcgcctgagctgtgccgccagcggattcaccttcggcagcaactatatgagctgggttcgccaagcacctggcaaaggcctggaatgggtgagcaccatcagcggcagcggcaccagcacctattatgccgatagcttgaaaggccgctttaccatcagccgcgataacagcaaaaacaccctgtatctgcagatgaacagcctgcgcgccgaggacaccgcagtctactactgtgcccgcggcatgtggggcatggatgtgtggggacaaggtactctggtgaccgtgagcagc

SEQ ID NO: 314 - DNA, 312 bp, synthetic construct
  source 1..312: mol_type = other DNA
cagagcgtgctgacccagcctcctagcgcctccggtacaccaggacagcgcgtgactattagctgtaccggcaaacatcggcacaccgtgaactggtaccagctactgcctggaactgcacctaagctgctgatctatctggatagcgaacgccctagcggcgtacctgatcgctttagcggtagcaaatcaggcaccagcgccagcctggccatcagcggccttcgctccgaagatgaagccgattattattgtcagagctatgatagcagcagcgtggtgtttggtggcggtaccaagctgaccgtgctg

SEQ ID NO: 315 - protein, 116 aa, synthetic construct
RVQLLESGGGLVQPGGSLRLSCAASGFTFGSNYMSWVRQAPGKGLEWVSTISGSGTSTYYADSLKGRFTISRDNSKNTLYLQMNSLRAEDTAVYYCARGMWGMDVWGQGTLVTVSS

SEQ ID NO: 316 - protein, 104 aa, synthetic construct
QSVLTQPPSASGTPGQRVTISCTGKHRHTVNWYQLLPGTAPKLLIYLDSERPSGVPDRFSGSKSGTSASLAISGLRSEDEADYYCQSYDSSSVVFGGGTKLTVL

SEQ ID NO: 317 - DNA, 351 bp, synthetic construct
  source 1..351: mol_type = other DNA
cgagtgcagctgctggaaagtggaggtggactggtgcagcctggcggcagcctgcgcctgagctgtgccgccagcggattcaccttcagcagctatgccatgcattgggttcgccaagcacctggcaaaggcctggaatgggtgagcagcatcagcggcggcggctatggcacctattatgccgatagcgtgaaaggccgctttaccatcagccgcgataacagcaaaaacaccctgtatctgcagatgaacagcctgcgcgccgaggacaccgcagtctactactgtgcccgcagcaccgtgtgggcctttgatatctggggacaaggtactctggtgaccgtgagcagc

SEQ ID NO: 318 - DNA, 321 bp, synthetic construct
  source 1..321: mol_type = other DNA
cagagcgtgctgacccagcctcctagcgcctccggtacaccaggacagcgcgtgactattagctgtagcggcaacaacatcggcagcaaaagcgtgcattggtaccagcaactgcctggaactgcacctaagctgctgatctatgatgtgagcaaacgccctagcgagcgtcctgatcgctttagcggtagcaaatcaggcaccagcgccagtctggccatcagcgaccttcgctccgaagatgaagccgattattattgtcagagctttgatagcagcggcacctggatctttggtggcggtaccaagctgaccgtgctg

SEQ ID NO: 319 - protein, 117 aa, synthetic construct
RVQLLESGGGLVQPGGSLRLSCAASGFTFSSYAMHWVRQAPGKGLEWVSSISGGGYGTYYADSVKGRFTISRDNSKNTLYLQMNSLRAEDTAVYYCARSTVWAFDIWGQGTLVTVSS

SEQ ID NO: 320 - protein, 107 aa, synthetic construct
QSVLTQPPSASGTPGQRVTISCSGNNIGSKSVHWYQQLPGTAPKLLIYDVSKRPSERPDRFSGSKSGTSASLAISDLRSEDEADYYCQSFDSSGTWIFGGGTKLTVL

SEQ ID NO: 321 - DNA, 357 bp, synthetic construct
  source 1..357: mol_type = other DNA
gaggtgcagctgttggagtctggtggaggcttggtacagcctggaggttctcttcgcctctcctgtgcagcctccggattcactttcagcagctacggtatgcattgggtcagacaggcaccaggtaagggactggagtgggtctctgcaattagcggtagcggtggtagcacttactacgcagacagcgtgaagggtcgcttcaccatctcacgcgacaactccaagaacaccctgtacctgcagatgaacagccttcgcgcagaggacactgccgtgtattactgcgcagtcagtggtgcaggtcgtggtttcttcgactactggggacaaggtactctggtcactgtctcctca

SEQ ID NO: 322 - DNA, 327 bp, synthetic construct
  source 1..327: mol_type = other DNA
cagtctgtgctgactcagccaccttcagcatctggtactccaggtcagcgcgtcaccatcagctgcagcggtagcagcagcaacattggtagcaactacgtgtactggtatcagcaactcccaggcaccgctcctaagctcctgatttacgaggacaacaagcgtcctagtggtgtgcctgatcgcttttctgggtccaagtctggcacctcagcctctctggctatcagtggacttcgctccgaggacgaggctgactattactgcagcagctacactagcagcagcactgtgatcttcggcggtgggaccaaactgaccgtccta

SEQ ID NO: 323 - protein, 119 aa, synthetic construct
EVQLLESGGGLVQPGGSLRLSCAASGFTFSSYGMHWVRQAPGKGLEWVSAISGSGGSTYYADSVKGRFTISRDNSKNTLYLQMNSLRAEDTAVYYCAVSGAGRGFFDYWGQGTLVTVSS

SEQ ID NO: 324 - protein, 109 aa, synthetic construct
QSVLTQPPSASGTPGQRVTISCSGSSSNIGSNYVYWYQQLPGTAPKLLIYEDNKRPSGVPDRFSGSKSGTSASLAISGLRSEDEADYYCSSYTSSSTVIFGGGTKLTVL

SEQ ID NO: 325 - DNA, 351 bp, synthetic construct
  source 1..351: mol_type = other DNA
gaggtgcagctgttggagtctggtggaggcttggtacagcctggaggttctcttcgcctctcctgtgcagcctccggattcactttcagccgctacgcaatgagctgggtcagacaggcaccaggtaagggactggagtgggtctctgcaattagcggtagcggtggtagcacttactacgcagacagcgtgaagggtcgcttcaccatctcacgcgacaactccaagaacaccctgtacctgcagatgaacagccttcgcgcagaggacactgccgtgtattactgcgcacgtagcagccagggtatcttcgacatctggggacaaggtactctggtcactgtctcctca

SEQ ID NO: 326 - DNA, 324 bp, synthetic construct
  source 1..324: mol_type = other DNA
cagtctgtgctgactcagccaccttcagcatctggtactccaggtcagcgcgtcaccatcagctgcagtggtaacaatatcggtactagacgcgtgcattggtatcagcaactcccagacaccgctcctaagctcctgatttacagtaagaacaaccgtcctagtggtgtgcctgatcgcttttctgggtccaagtctggcacctcagcctctctggctatcagtggacttcgctccgaggacgaggctgactattactgcgcagcatgggacgacagcctgagcggtcctgtgttcggcggtgggaccaaactgaccgtccta

SEQ ID NO: 327 - protein, 117 aa, synthetic construct
EVQLLESGGGLVQPGGSLRLSCAASGFTFSRYAMSWVRQAPGKGLEWVSAISGSGGSTYYADSVKGRFTISRDNSKNTLYLQMNSLRAEDTAVYYCARSSQGIFDIWGQGTLVTVSS

SEQ ID NO: 328 - protein, 108 aa, synthetic construct
QSVLTQPPSASGTPGQRVTISCSGNNIGTRRVHWYQQLPDTAPKLLIYSKNNRPSGVPDRFSGSKSGTSASLAISGLRSEDEADYYCAAWDDSLSGPVFGGGTKLTVL

SEQ ID NO: 329 - DNA, 354 bp, synthetic construct
  source 1..354: mol_type = other DNA
gaggtgcagctgttggagtctggtggaggcttggtacagcctggaggttctcttcgcctctcctgtgcagcctccggattcactttcagcagctacgcaatgagctgggtcagacaggcaccaggtaagggactggagtgggtctctgcaattagcggtagcggtggtagcacttactacgcagacagcgtgaagggtcgcttcaccatctcacgcaacaactccaagaacaccctgtacctgcagatgaacagccttcgcgcagaggacactgccgtgtattactgcgcacgtagcggtcgttacgcagacttgacatctgggggacaaggtactctggtcactgtctcctca

SEQ ID NO: 330 - DNA, 327 bp, synthetic construct
  source 1..327: mol_type = other DNA
cagtctgtgctgactcagccaccttcagcatctggtactccaggtcagcgcgtcaccatcagctgcagcggtagcaacagcaacatcggtaacaactacgtgagctggtatcagcaactcccagacacccctcctaagctcctgatttacgacaacaacaagcgtcctagtggtgtgcctgatcgcttttctgggtccaagtctggcacctcagcctctctggctatcagtggacttcgctccgaggacgaggctgactattactgcagcagctacactagcagcagcactgtgatgttcggcggtgggaccaaactgaccgtccta

SEQ ID NO: 331 - protein, 118 aa, synthetic construct
EVQLLESGGGLVQPGGSLRLSCAASGFTFSSYAMSWVRQAPGKGLEWVSAISGSGGSTYYADSVKGRFTISRNNSKNTLYLQMNSLRAEDTAVYYCARSGRYADLTSGGQGTLVTVSS

SEQ ID NO: 332 - protein, 109 aa, synthetic construct
QSVLTQPPSASGTPGQRVTISCSGSNSNIGNNYVSWYQQLPDTPPKLLIYDNNKRPSGVPDRFSGSKSGTSASLAISGLRSEDEADYYCSSYTSSSTVMFGGGTKLTVL

SEQ ID NO: 333 - DNA, 351 bp, synthetic construct
  source 1..351: mol_type = other DNA
gaggtgcagctgttggagtctggtggaggcttggtacagcctggaggttctcttcgcctctcctgtgcagcctccggattcactttcagcagctactactggagctgggtcagacaggcaccaggtaagggactggagtgggtctctgcaattagcggtagcggtggtagcacttactacgcagacagcgtgaagggtcgcttcaccatctcacgcgacaactccaagaacaccctgtacctgcagatgaacagccttcgcgcagaggacactgccgtgtattactgcgcacgtatcgacgtgtacggtttcgacatctggggacaaggtactctggtcactgtctcctca

SEQ ID NO: 334 - DNA, 327 bp, synthetic construct
  source 1..327: mol_type = other DNA
cagtctgtgctgactcagccaccttcagcatctggtactccaggtcagcgcgtcaccatcagctgcagcggtagcactagcaacatcggtactaactacgtgtactggtatcagcaactcccaggcaccgctcctaagctcctgatttacgacaacaacaaccgtcctagtggtgtgcctgatcgcttttctgggtccaagtctggcacctcagcctctctggctatcagtggacttcgctccgaggacgaggctgactattactgccagacttgggacagcagcactgacgtagtgttcggcggtgggaccaaactgaccgtccta

SEQ ID NO: 335 - protein, 117 aa, synthetic construct
EVQLLESGGGLVQPGGSLRLSCAASGFTFSSYYWSWVRQAPGKGLEWVSAISGSGGSTYYADSVKGRFTISRDNSKNTLYLQMNSLRAEDTAVYYCARIDVYGFDIWGQGTLVTVSS

SEQ ID NO: 336 - protein, 109 aa, synthetic construct
QSVLTQPPSASGTPGQRVTISCSGSTSNIGTNYVYWYQQLPGTAPKLLIYDNNNRPSGVPDRFSGSKSGTSASLAISGLRSEDEADYYCQTWDSSTDVVFGGGTKLTVL

SEQ ID NO: 337 - DNA, 348 bp, synthetic construct
  source 1..348: mol_type = other DNA
gaggtgcagctgttggagtctggtggaggcttggtacagcctggaggttctcttcgcctctcctgtgcagcctccggattcactttcagcagctacggtatgcattgggtcagacaggcaccaggtaagggactggagtgggtctctgcaattagcggtagcggtggtagcacttactacgcagacagcgtgaagggtcgcttcaccatctcacgcgacaactccaagaacaccctgtacctgcagatgaacagccttcgcgcagaggacactgccgtgtattactgcgcaagcggttacggtctgatggacgtgtggggacaaggtactctggtcactgtctcctca

SEQ ID NO: 338 - DNA, 324 bp, synthetic construct
  source 1..324: mol_type = other DNA
tctgtgctgactcagccaccttcagcatctggtactccaggtcagcgcgtcaccatcagctgcactcgtagcagcggtatcatcgcaagcaactacgtgcagtggtatcagcaactcccaggcaccgctcctaagctcctgatttaccgcaacaaccagcgccctagtggtgtgcctgatcgcttttctgggtccaagtctggcacctcagcctctctggctatcagtggacttcgctccgaggacgaggctgactattactgcagcagctacgcaggtaacaacaacctggtgttcggcggtgggaccaaactgaccgtccta

SEQ ID NO: 339 - protein, 116 aa, synthetic construct
EVQLLESGGGLVQPGGSLRLSCAASGFTFSSYGMHWVRQAPGKGLEWVSAISGSGGSTYYADSVKGRFTISRDNSKNTLYLQMNSLRAEDTAVYYCASGYGLMDVWGQGTLVTVSS

SEQ ID NO: 340 - protein, 109 aa, synthetic construct
QSVLTQPPSASGTPGQRVTISCTRSSGIIASNYVQWYQQLPGTAPKLLIYRNNQRPSGVPDRFSGSKSGTSASLAISGLRSEDEADYYCSSYAGNNNLVFGGGTKLTVL

SEQ ID NO: 341 - DNA, 348 bp, synthetic construct
  source 1..348: mol_type = other DNA
cgagtgcagctgctggaaagtggaggtggactggtgcagcctggcggcagcctgcgcctgagctgtgccgccagcggattcaccttcagcacctatggcatgcattgggttcgccaagcacctggcaaaggcctggaatgggtgagcgccatcagcggcagcggcggcagcacctattatgccgatagcgtgaaaggccgctttaccatcagccgcgataacagcaaaaacaccctgtatctgcagatgaacagcctgcgcgccgaggacaccgcagtctactactgtgcccgcggcctgagcggccttgattattggggacaaggtactctggtgaccgtgagcagc

SEQ ID NO: 342 - DNA, 321 bp, synthetic construct
  source 1..321: mol_type = other DNA
gaaatcgtgctgacccagagccctggcaccctgagcctgagccctggcgaacgcgcaacactgtcatgccgctccagccagggcatcaccaactatctggcctggtatcagcagaaaccaggtcaggctccacgtctgctgatctatgatgccagcaaccgcgccaccggcatccctgatcgcttctcaggatctggaagcggtaccgattttaccctgaccatcagccgcctggaacctgaggactttgccgtgtattattgtcagcagagctatagcacccctctgaccttcggtcagggcactaaagtggaaatcaaa

SEQ ID NO: 343 - protein, 116 aa, synthetic construct
RVQLLESGGGLVQPGGSLRLSCAASGFTFSTYGMHWVRQAPGKGLEWVSAISGSGGSTYYADSVKGRFTISRDNSKNTLYLQMNSLRAEDTAVYYCARGLSGLDYWGQGTLVTVSS

SEQ ID NO: 344 - protein, 107 aa, synthetic construct
EIVLTQSPGTLSLSPGERATLSCRSSQGITNYLAWYQQKPGQAPRLLIYDASNRATGIPDRFSGSGSGTDFTLTISRLEPEDFAVYYCQQSYSTPLTFGQGTKVEIK

SEQ ID NO: 345 - DNA, 348 bp, synthetic construct
  source 1..348: mol_type = other DNA
cgagtgcagctgctggaaagtggaggtggactggtgcagcctggcggcagcctgcgcctgagctgtgccgccagcggattcaccttcagcagctatgccatgcattgggttcgccaagcacctggcaaaggcctggaatgggtgagcgccatcagcggcagcggcggcgatacctatcatgccgatagcgtgaaaggccgctttaccatcagccgcgataacagcaaaaacaccctgtatctgcagatgaacagcctgcgcgccgaggacaccgcagtctactactgtacccgcggcctgagcggctttgattattggggacaaggtactctggtgaccgtgagcagc

SEQ ID NO: 346 - DNA, 321 bp, synthetic construct
  source 1..321: mol_type = other DNA
gaaatcgtgctgacccagagccctggcaccctgagcctgagccctggcgaacgcgcaacactgtcatgccgcgccagccagagcatcagcagctatctgaactggtatcagcagaaaccaggtcaggctccacgtctgctgatctatgatgccagcaaccgcgcccctggcatccctgatcgcttctcaggatctggaagcggtaccgattttaccctgaccatcagccgcctggaacctgaggactttgccgtgtattattgtcagcagagctatagcatccctatcaccttcggtcagggcactaaagtggaaatcaaa

SEQ ID NO: 347 - protein, 116 aa, synthetic construct
RVQLLESGGGLVQPGGSLRLSCAASGFTFSSYAMHWVRQAPGKGLEWVSAISGSGGDTYHADSVKGRFTISRDNSKNTLYLQMNSLRAEDTAVYYCTRGLSGFDYWGQGTLVTVSS

SEQ ID NO: 348 - protein, 110 aa, synthetic construct
EIVLTQSPGTLSLSPGERATLSCRASQSISSYLNWYQQKPGQAPRLLIYDASNRAPGIPDRFSGSGSGTDFTLTISRLEPEDFAVYYCQQSYSIPITFGQGTKVEIKFSD

SEQ ID NO: 349 - DNA, 348 bp, synthetic construct
  source 1..348: mol_type = other DNA
cgagtgcagctgctggaaagtggaggtggactggtgcagcctggcggcagcctgcgcctgagctgtgccgccagcggattcaccttcagcgattatgccatgagctgggttcgccaagcacctggcaaaggcctggaatgggtgagcagcatcagcagcagcagcagctatatctactataccgatagcgtgaaaggccgctttaccatcagccgcgataacagcaaaaacaccctgtatctgcagatgaacagcctgcgcgccgaggacaccgcagtctactactgtgcccgcggcggctatggctttgattattggggacaaggtaccctggtgaccgtgagcagc

SEQ ID NO: 350 - DNA, 321 bp, synthetic construct
  source 1..321: mol_type = other DNA
gaaatcgtgctgacccagagccctggcaccctgagcctgagccctggcgaacgcgcaacactgtcatgccgcgccagccagagcatcagcagctatctgaactggtatcagcagaaaccaggtcaggctccacgtctgctgatctatagcgccagcagccgcccacagggcatccccgatcgcttctcaggatctggaagcggtaccgattttaccctgaccatcagccgcctggaacctgaggactttgccgtgtattattgtcagcagtatgatgatctgccttttaccttcggtcagggcactaaagtggaaatcaaa

SEQ ID NO: 351 - protein, 116 aa, synthetic construct
RVQLLESGGGLVQPGGSLRLSCAASGFTFSDYAMSWVRQAPGKGLEWVSSISSSSSYIYYTDSVKGRFTISRDNSKNTLYLQMNSLRAEDTAVYYCARGGYGFDYWGQGTLVTVSS

SEQ ID NO: 352 - protein, 107 aa, synthetic construct
EIVLTQSPGTLSLSPGERATLSCRASQSISSYLNWYQQKPGQAPRLLIYSASSRPQGIPDRFSGSGSGTDFTLTISRLEPEDFAVYYCQQYDDLPFTFGQGTKVEIK

SEQ ID NO: 353 - DNA, 346 bp, synthetic construct
  source 1..346: mol_type = other DNA
gaagtgcagctgctggaaagtggaggtggactggtgcagcctggcggcagcctgcgcctgagctgtgccgccagcggattcaccttcagcaactttgcgatcgcctgggttcgccaagcacctggcaaaggcctggaatgggtgagcgccatcagcggccgcggcaccagcacctattatgccgatagcgtgaaaggccgctttaccatcagccgcgataacagcaaaaacaccctgtatctgcagatgaacagcctgcgcgccgaggacaccgcagtctactactgtgcccgcggcgtgagcggctttgatagctggggacaaggtactctggtgaccgtgagca

SEQ ID NO: 354 - DNA, 321 bp, synthetic construct
  source 1..321: mol_type = other DNA
gaaatcgtgctgacccagagccctggcaccctgagcctgagccctggcgaacgcgcaacactgtcatgccgcgccagccagagcatcagcagccatctggcctggtatcagcagaaaccaggtcaggctccacgtctgctgatctatgataccagcaaccgcgccaccggcatccctgatcgcttctcaggatctgggagcggtaccgattttaccctgaccatcagccgcctggaacctgaggactttgccgtgtactattgtcagcagagctatagcaccccttttaccttcggtcagggcactaaagtggaaatcaaa

SEQ ID NO: 355 - protein, 116 aa, synthetic construct
EVQLLESGGGLVQPGGSLRLSCAASGFTFSNFAIAWVRQAPGKGLEWVSAISGRGTSTYYADSVKGRFTISRDNSKNTLYLQMNSLRAEDTAVYYCARGVSGFDSWGQGTLVTVSS

SEQ ID NO: 356 - protein, 107 aa, synthetic construct
EIVLTQSPGTLSLSPGERATLSCRASQSISSHLAWYQQKPGQAPRLLIYDTSNRATGIPDRFSGSGSGTDFTLTISRLEPEDFAVYYCQQSYSTPFTFGQGTKVEIK

SEQ ID NO: 357 - DNA, 349 bp, synthetic construct
  source 1..349: mol_type = other DNA
cgagtgcagctgctggaaagtggaggtggactggtgcagcctggcggcagcctgcgcctgagctgtgccgccagcggattcaccttcagcagctatgccatgcattgggttcgccaagcacctggcaaaggcctggaatgggtgagcgccatcaacggcagcggcggcagcacctattatgccgatagcgtgaaaggccgctttaccatcagccgcgataacagcaaaaacaccctgtatctgcagacgaacagcctgcgcgccgaggacaccgcagtctactactgtgcccgcggcctgcagggctttgattattggggacaaggtactctggtgaccgtgagcagca

SEQ ID NO: 358 - DNA, 321 bp, synthetic construct
  source 1..321: mol_type = other DNA
gaaatcgtgctgacccagagccctggcaccctgagcctgagccctggcgaacgcgcaacactgtcatgccaggccagccaggatatcaccaactatctgaactggtatcagcagaaaccaggtcaggctccacgtctgctgatctatgatgccagcagcctggaaaccggcatccctgatcgtttctcaggatctggaagcggtaccgattttaccctgaccatcagccgcctggaacctgaggactttgccgtgtattattgtcagcagagctatagcacccctatcaccttcggtcagggcactaaagtggaaatcaaa

SEQ ID NO: 359 - protein, 116 aa, synthetic construct
RVQLLESGGGLVQPGGSLRLSCAASGFTFSSYAMHWVRQAPGKGLEWVSAINGSGGSTYYADSVKGRFTISRDNSKNTLYLQTNSLRAEDTAVYYCARGLQGFDYWGQGTLVTVSS

SEQ ID NO: 360 - protein, 107 aa, synthetic construct
EIVLTQSPGTLSLSPGERATLSCQASQDITNYLNWYQQKPGQAPRLLIYDASSLETGIPDRFSGSGSGTDFTLTISRLEPEDFAVYYCQQSYSTPITFGQGTKVEIK

SEQ ID NO: 361 - DNA, 349 bp, synthetic construct
  source 1..349: mol_type = other DNA
cgagtgcagctgctggaaagtggaggtggactggtgcagcctggcggcagcctgcgcctgagctgtgccgccagcggattcaccttcagcagctatgccatgagctgggttcgccaagcacctggcaaaggcctggaatgggtgagcgccatcaacggcagcggcggcagcaccctgtatgccgatagcgtgaaaggccgctttaccatcagccgcgataacagcaaaaacaccctgtatctgcagatgaacagcctgcgcgccgaggacaccgcagtctactactgtgcccgcggcgtgagcggctttgatagctggggacaaggtactctggtgaccgtgagcagcg

SEQ ID NO: 362 - DNA, 321 bp, synthetic construct
  source 1..321: mol_type = other DNA
gaaatcgtgctgacccagagccctggcaccctgagcctgagccctggcgaacgcgcaacactgtcatgccgcatcagccagagcatcagcagctatctgaactggtatcagcagaaaccaggtcaggctccacgtctgctgatctatgatgccagcctgcgcgccaccggcatccctgatcgcttctcaggatctggaagcggtaccgattttaccctgaccatcagccgcctggaacctgaggactttgccgtgtattattgtcagcagagctataaaacccctatcaccttcggtcagggcactaaagtggaaatcaaa

SEQ ID NO: 363 - protein, 116 aa, synthetic construct
RVQLLESGGGLVQPGGSLRLSCAASGFTFSSYAMSWVRQAPGKGLEWVSAINGSGGSTLYADSVKGRFTISRDNSKNTLYLQMNSLRAEDTAVYYCARGVSGFDSWGQGTLVTVSS

SEQ ID NO: 364 - protein, 107 aa, synthetic construct
EIVLTQSPGTLSLSPGERATLSCRISQSISSYLNWYQQKPGQAPRLLIYDASLRATGIPDRFSGSGSGTDFTLTISRLEPEDFAVYYCQQSYKTPITFGQGTKVEIK

SEQ ID NO: 365 - DNA, 349 bp, synthetic construct
  source 1..349: mol_type = other DNA
gaagtgcagctgctggaaagtggaggtggactggtgcagcctggcggcagcctgcgcctgagctgtgccgccagcggattcaccttcagcagctattattggagctgggttcgccaagcacctggcaaaggcctggaatgggtgagcaccatcaccggcagcggcggcagcaccgattatgccaacagcgtgaaaggccgctttaccatcagccgcgataacagcaaaaacaccctgtatctgcagatgaacagcctgcgcgccgaggacaccgcagtctactactgtgccaccggcggcggcatctttgactattggggacaaggtactctggtgaccgtgagcagcg

SEQ ID NO: 366 - DNA, 321 bp, synthetic construct
  source 1..321: mol_type = other DNA
gaaatcgtgctgacccagagccctggcaccctgagcctgagccctggcgaacgcgcaacactgtcatgccaggccagccagaccatcagcaactatctgaactggtatcagcagaaaccaggtcaggctccacgtctgctgatctatgatgccagcaaccgcgccaccggcatccctgatcgcttctcaggatctggaagcggtaccgattttaccctgaccatcagccgcctggaacctgaggactttgccgtgtattattgtcagcagtacaacagctatcctcctagcttcggtcagggcactaaagtggaaatcaaa

SEQ ID NO: 367 - protein, 116 aa, synthetic construct
EVQLLESGGGLVQPGGSLRLSCAASGFTFSSYYWSWVRQAPGKGLEWVSTITGSGGSTDYANSVKGRFTISRDNSKNTLYLQMNSLRAEDTAVYYCATGGGIFDYWGQGTLVTVSS

SEQ ID NO: 368 - protein, 107 aa, synthetic construct
EIVLTQSPGTLSLSPGERATLSCQASQTISNYLNWYQQKPGQAPRLLIYDASNRATGIPDRFSGSGSGTDFTLTISRLEPEDFAVYYCQQYNSYPPSFGQGTKVEIK

SEQ ID NO: 369 - DNA, 352 bp, synthetic construct
  source 1..352: mol_type = other DNA
cgagtgcagctgctggaaagtggaggtggactggtgcagcctggcggcagcctgcgcctgagctgtgccgccagcggattcaccttcagcgattatcatatgcattgggttcgccaagcacctggcaaaggcctggaatgggtgagcaccatcagcagcagcggcggctatacctattatgccgaaagcgtgaaaagccgctttaccatcagccgcgataacagcaaaaacaccctgtatctgcagatgaacagcctgcgcgccgaggacaccgcagtctactactgtgcccgatcgatacgcctgcctctggattattggggacaaggtactctggtgaccgtgagcagca

SEQ ID NO: 370 - DNA, 321 bp, synthetic construct
  source 1..321: mol_type = other DNA
cagagcgtgctgacccagcctcctagcgcctccggtacaccaggacagcgcgtgactattagctgtagcggcaacaacatcggcagcaaaggcgtgcattggtatcagcaactgcctggaactgcacctaagctgctgatctatgaagatagcaaacgccctagcggcgtgcgtgatcgctttagcggtagcaaatcaggcaccagcgccagcctggccatcagcggccttcgctccgaagatgaagccgattattattgtcagagctatgatagcaccaaaggcgtggtgtttggtggcggtaccaagctgaccgtgctg

SEQ ID NO: 371 - protein, 117 aa, synthetic construct
RVQLLESGGGLVQPGGSLRLSCAASGFTFSDYHMHWVRQAPGKGLEWVSTISSSGGYTYYAESVKSRFTISRDNSKNTLYLQMNSLRAEDTAVYYCARSIRLPLDYWGQGTLVTVSS

SEQ ID NO: 372 - protein, 107 aa, synthetic construct
QSVLTQPPSASGTPGQRVTISCSGNNIGSKGVHWYQQLPGTAPKLLIYEDSKRPSGVRDRFSGSKSGTSASLAISGLRSEDEADYYCQSYDSTKGVVFGGGTKLTVL

SEQ ID NO: 373 - DNA, 348 bp, synthetic construct
  source 1..348: mol_type = other DNA
gaggtgcagctgttggagtctggtggaggcttggtacagtctggaggttctcttcgcctctcctgtgcagcctccggattcactttcagcagctacggtatgcattgggtcagacaggcaccaggtaagggactggagtgggtctctgcaattagcggtagcggtggtagcacttactacgcagacagcgtgaagggtcgcttcaccatctcacgcgacaactccaagaacaccctgtacctgcagatgaacagccttcgcgcagaggacactgccgtgtattactgcgtgcgtggttacggtgcaatggacgtgtggggacaaggtactctggtcactgtctcctca

SEQ ID NO: 374 - DNA, 327 bp, synthetic construct
  source 1..327: mol_type = other DNA
cagtctgtgctgactcagccaccttcagcatctggtactccaggtcagcgcgtcaccatcagctgcactcgtagcagcggtagcatcgcaagcaactacgtgcagtggtatcagcaactcccaggcaccgctcctaagctcctgatttaccgcaacaaccagcgccctagtggtgtgcctgatcgcttttctgggtccaagtctggcacctcagcctctctggctatcagtggacttcgctccgaggacgaggctgactattactgcagcagctacactactagcagcactctggtgttcggcggtgggaccaaactgaccgtccta

SEQ ID NO: 375 - protein, 116 aa, synthetic construct
EVQLLESGGGLVQSGGSLRLSCAASGFTFSSYGMHWVRQAPGKGLEWVSAISGSGGSTYYADSVKGRFTISRDNSKNTLYLQMNSLRAEDTAVYYCVRGYGAMDVWGQGTLVTVSS

SEQ ID NO: 376 - protein, 109 aa, synthetic construct
QSVLTQPPSASGTPGQRVTISCTRSSGSIASNYVQWYQQLPGTAPKLLIYRNNQRPSGVPDRFSGSKSGTSASLAISGLRSEDEADYYCSSYTTSSTLVFGGGTKLTVL

SEQ ID NO: 377 - DNA, 348 bp, synthetic construct
  source 1..348: mol_type = other DNA
gaggtgcagctgttggagtctggtggaggcttggtacagcctggaggttctcttcgcctctcctgtgcagcctccggattcactttcagcagctacgcaatgcattgggtcagacaggcaccaggtaagggactggagtgggtctctgcaattagcggtagcggtggtagcacttactacgcagacagcgtgaagggtcgcttcaccatctcacgcgacaactccaagaacaccctgtacctgcagatgaacagccttcgcgcaaaggacactgccgtgtattactgcgcaagcggctacggtctgatggacgtatggggacaaggtactctggtcactgtctcctca

SEQ ID NO: 378 - DNA, 330 bp, synthetic construct
  source 1..330: mol_type = other DNA
cagtctgtgctgactcagccaccttcagcatctggtactccaggtcagcgcgtcaccatcagctgcactggtactagcagcgacgtgggtaactacaacctggtgagctggtatcagcaactcccaggcaccgctcctaagctcctgatttacagcaacaaccagcgccctagtggtgtgcctgatcgcttttctgggtccaagtctggcacctcagcctctctggctatcagtggacttcgctccgaggacgaggctgactattactgcagcagctacactggtagcaacgctctgttgttcggcggtgggaccaaactgaccgtccta

SEQ ID NO: 379 - protein, 116 aa, synthetic construct
EVQLLESGGGLVQPGGSLRLSCAASGFTFSSYAMHWVRQAPGKGLEWVSAISGSGGSTYYADSVKGRFTISRDNSKNTLYLQMNSLRAKDTAVYYCASGYGLMDVWGQGTLVTVSS

SEQ ID NO: 380 - protein, 110 aa, synthetic construct
QSVLTQPPSASGTPGQRVTISCTGTSSDVGNYNLVSWYQQLPGTAPKLLIYSNNQRPSGVPDRFSGSKSGTSASLAISGLRSEDEADYYCSSYTGSNALLFGGGTKLTVL

SEQ ID NO: 381 - DNA, 348 bp, synthetic construct
  source 1..348: mol_type = other DNA
gaggtgcagctgttggagtctggtggaggcttggtacagcctggaggttctcttcgcctctcctgtgcagcctccggattcactttcagcagctacgcaatgagctgggtcagacaggcaccaggtaagggactggagtgggtctctgcaattagcggtagcggtggtagcacttactacgcagacagcgtgaagggtcgcttcaccatctcacgcgacaactccaagaacaccctgtacctgcagatgaacagccttcgcgcagaggacactgccgtgtattactgcgcacgctggcattacagcttcgactactggggacaaggtactctggtcactgtctcctca

SEQ ID NO: 382 - DNA, 324 bp, synthetic construct
  source 1..324: mol_type = other DNA
cagtctgtgctgactcagccaccttcagcatctggtactccaggtcagcgcgtcaccatcagctgccgtggtaacaacatcggtagcaagcgtgtgcattggtatcagcaactcccaggcaccgctcctaagctcctgatttacagctacaaccaccgtcctagcggtgtgcctgatcgcttttctgggtccaagtctggcacctcagcctctctggctatcactggacttcgctccgaggacgaagctgactattactgcaacacttgggacgacagcctggagggtcctgtgttcggcggtgggaccaaactgaccgtccta

SEQ ID NO: 383 - protein, 116 aa, synthetic construct
EVQLLESGGGLVQPGGSLRLSCAASGFTFSSYAMSWVRQAPGKGLEWVSAISGSGGSTYYADSVKGRFTISRDNSKNTLYLQMNSLRAEDTAVYYCARWHYSFDYWGQGTLVTVSS

SEQ ID NO: 384 - protein, 108 aa, synthetic construct
QSVLTQPPSASGTPGQRVTISCRGNNIGSKRVHWYQQLPGTAPKLLIYSYNHRPSGVPDRFSGSKSGTSASLAITGLRSEDEADYYCNTWDDSLEGPVFGGGTKLTVL

SEQ ID NO: 385 - DNA, 352 bp, synthetic construct
  source 1..352: mol_type = other DNA
gaggtgcagctgttggagtctggtggaggcttggtacagcctggaggttctcttcgcctctcctgtgcagcctccggattcactttcagcggctacgcaatgagctgggtcagacaggcaccaggtaagggactggagtgggtctctgcaattagcggtagcggtggtagcacttactacgcagacagcgtgaagggtcgcttcaccatctcacgcgacaactccaagaacaccctgtacctgcagatgaacagccttcgcgcagaggacactgccgtgtattactgcgcacgtagtcctagcggtctgttcgactactggggacaaggtactctggtcactgtctcctcag

SEQ ID NO: 386 - DNA, 318 bp, synthetic construct
  source 1..318: mol_type = other DNA
cagtctgtgctgactcagccaccttcagcatctggtactccaggtcagcgcgtcaccatcagctgcggtggtaacaacatcggtagcaagcgtgtgcattggtatcagcaactcccaggcaccgctcctaagctcctgatttacaacactagcaacaagcatagcggtgtgcctgatcgcttttctgggtccaagtctggcacctcagcctctctggctatcagtggacttcgctccgaggacgaggctgactattactgcagcagctacctacagcagcactctctgttcggcggtgggaccaaactaaccgtccta

SEQ ID NO: 387 - protein, 117 aa, synthetic construct
EVQLLESGGGLVQPGGSLRLSCAASGFTFSGYAMSWVRQAPGKGLEWVSAISGSGGSTYYADSVKGRFTISRDNSKNTLYLQMNSLRAEDTAVYYCARSPSGLFDYWGQGTLVTVSS

SEQ ID NO: 388 - protein, 106 aa, synthetic construct
QSVLTQPPSASGTPGQRVTISCGGNNIGSKRVHWYQQLPGTAPKLLIYNTSNKHSGVPDRFSGSKSGTSASLAISGLRSEDEADYYCSSYLQQHSLFGGGTKLTVL

SEQ ID NO: 389 - DNA, 360 bp, synthetic construct
  source 1..360: mol_type = other DNA
gaggtgcagctgttggagtctggtggaggcttggtacagcctggaggttcctcttccgcctcctcctgtgcagcctccggattcactttcagcagctacgcaatgagctgggtcagacaggcaccaggtaagggactggagtgggtctctgcaattagcggtagcggtggtagcacttactacgcagacagcgtgaagggtcgcttcaccatctcacgcgacaactccaagaacaccctgtacctgcagatgaacagccttcgcgcagaggacactgccgtgtattactgcacacgtttcgtgggtgcaatcggtgcattcgactactggggacaaggtactctggtcactgtctcctca

SEQ ID NO: 390 - DNA, 324 bp, synthetic construct
  source 1..324: mol_type = other DNA
cagtctgtgctgactcagccaccttcagcatctggtactccaggtcagcgcgtcaccatcagctgcagtggtaacaacatcggtagccgtagcgtgcattggtatcagcaactcccaggcaccgctcctaagctcctgatttaccgcaacaaccagcgccctagtggtgtgcctgatcgcttttctgggtccaagtctggcacctcagcctctctggctatcagtggacttcgctccgaggacgaggctgactattactgcgcagcatgggacgacagcctgagcggtcctgtgttcggcggtgggaccaaactgaccgtccta

SEQ ID NO: 391 - protein, 120 aa, synthetic construct
EVQLLESGGGLVQPGGSSSASSCAASGFTFSSYAMSWVRQAPGKGLEWVSAISGSGGSTYYADSVKGRFTISRDNSKNTLYLQMNSLRAEDTAVYYCTRFVGAIGAFDYWGQGTLVTVSS

SEQ ID NO: 392 - protein, 108 aa, synthetic construct
QSVLTQPPSASGTPGQRVTISCSGNNIGSRSVHWYQQLPGTAPKLLIYRNNQRPSGVPDRFSGSKSGTSASLAISGLRSEDEADYYCAAWDDSLSGPVFGGGTKLTVL

SEQ ID NO: 393 - DNA, 363 bp, synthetic construct
  source 1..363: mol_type = other DNA
gaggtgcagctgttggagtctggtggaggcttggtacagcctggaggttctcttcgcctctcctgtgcagcctccggattcactttcagccattacgcaatgagctgggtcagacaggcaccaggtaagggactggagtgggtctctgcaattagcggtagcggtggtagcacttactacgcagacagcgtgaagggtcgcttcaccatctcacgcgacaactccaagaacaccctgtacctgcagatgaacagccttcgcgcagaggacactgccgtgtattactgcgcacgtggttgggacagccctactctgacatacttcgacagctggggacaaggtactctggtcactgtctcctca

SEQ ID NO: 394 - DNA, 330 bp, synthetic construct
  source 1..330: mol_type = other DNA
cagtctgtgctgactcagccaccttcagcatctggtactccaggtcagcgcgtcaccatcagctgcagcggtactagcagcaacatcggtaacaacgacgtgagctggtatcagcaactcccaggcaccgctcctaagctcctgatttaccaggacactaagcgtcctagcggtgtgcctgatcgcttttctgggtccaagtctggcacctcagcctctctggctatcagtggacttcgctccgaggacgaggctgactattactgcgcagcatgggacgacagcctgagcggtcctgtgttcggcggtgggaccaaactgaccgtccta

SEQ ID NO: 395 - protein, 121 aa, synthetic construct
EVQLLESGGGLVQPGGSLRLSCAASGFTFSHYAMSWVRQAPGKGLEWVSAISGSGGSTYYADSVKGRFTISRDNSKNTLYLQMNSLRAEDTAVYYCARGWDSPTLTYFDSWGQGTLVTVSS

SEQ ID NO: 396 - protein, 110 aa, synthetic construct
QSVLTQPPSASGTPGQRVTISCSGTSSNIGNNDVSWYQQLPGTAPKLLIYQDTKRPSGVPDRFSGSKSGTSASLAISGLRSEDEADYYCAAWDDSLSGPVFGGGTKLTVL

SEQ ID NO: 397 - DNA, 348 bp, synthetic construct
  source 1..348: mol_type = other DNA
gaggtgcagctgttggagtctggtggaggcttggtacagcctggaggttctcttcgcctctcctgtgcagcctccggattcactttcagcagctacggtatgcattgggtcagacaggcaccaggtaagggactggagtgggtctctgcaatcagcggtagcggtggttacacttactacgcagacagcgtgaagggtcgcttcaccatctcacgcgacaactccaagaacaccctgtacctgcagatgaacagccttcgcgcagaggacactgccgtgtattactgcgcacgctggcattacagcttcgactactggggacaaggtactctggtcactgtctcctca

SEQ ID NO: 398 - DNA, 324 bp, synthetic construct
  source 1..324: mol_type = other DNA
cagtctgtgctgactcagccaccttcagcatctggtactccaggtcagcgcgtcaccatcagctgcagcggtagcagcagcaacatcggtaacaactacgtgagctggtatcagcaactcccaggcaccgctcctaagctcctgatttaccgcaacaaccagcgccctagtggtgtgcctgatcgcttttctgggtccaagtctggcacctcagcctctctggctatcagtggacttcgctccgaggacgaggctgactattactgccagagctacgacaacagcaacgtgctgttcggcggtgggaccaaactgaccgtccta

SEQ ID NO: 399 - protein, 116 aa, synthetic construct
EVQLLESGGGLVQPGGSLRLSCAASGFTFSSYGMHWVRQAPGKGLEWVSAISGSGGYTYYADSVKGRFTISRDNSKNTLYLQMNSLRAEDTAVYYCARWHYSFDYWGQGTLVTVSS

SEQ ID NO: 400 - protein, 108 aa, synthetic construct
QSVLTQPPSASGTPGQRVTISCSGSSSNIGNNYVSWYQQLPGTAPKLLIYRNNQRPSGVPDRFSGSKSGTSASLAISGLRSEDEADYYCQSYDNSNVLFGGGTKLTVL

SEQ ID NO: 401 - DNA, 489 bp, synthetic construct
  source 1..489: mol_type = other DNA
ggctattttcctctgagccaccccatgaccgtggcgggccccgtggggggatccctgagtgtgcagtgtcgctatgagaaggaacacaggaccctcaacaaattctggtgcagaccaccacagattctccgatgtgacaagattgtggagaccaaagggtcagcagggaaaaggaatggccgagtgtccatcagggacagtcctgcaaacctcagcttcacagtgaccctggagaatctcacagaggaggacgcaggcacctactggtgtggggtggatacaccgtggctccgagactttcatgatcccattgtcgaggttgaggtgtccgtgttcccggccgggacgaccacagcctccagcccccagagctccatgggcacctcaggtcctcccacgaagctgcccgtgcacacctggcccagcgtgaccagaaaggacagccccgaacccagcccacaccctggctccctgttcagcaatgtccgc

SEQ ID NO: 402 - protein, 163 aa, synthetic construct
GYFPLSHPMTVAGPVGGSLSVQCRYEKEHRTLNKFWCRPPQILRCDKIVETKGSAGKRNGRVSIRDSPANLSFTVTLENLTEEDAGTYWCGVDTPWLRDFHDPIVEVEVSVFPAGTTTASSPQSSMGTSGPPTKLPVHTWPSVTRKDSPEPSPHPGSLFSNVR